European Patent Application EP 4 209 594 A1, published July 12, 2023. Title: 一种表达盒、载体及其在昆虫细胞中制备重组腺相关病毒的应用. Applicant: 武汉枢密脑科学技术有限公司. The sequence listing filed with the application follows.

SEQUENCE LISTING (14 sequences)

SEQ ID NO: 1 - DNA, 110 bp, AcMNPV
  Promoter p10
gacctttaattcaacccaacacaatatattatagttaaataagaattattatcaaatcatttgtatattaattaaaatactatactgtaaattacattttatttacaatc

SEQ ID NO: 2 - DNA, 226 bp, Artificial Sequence
  Intron1+Intron2
gtaagtattcattgtaaatctgatattatttgtattattatacctacctaatttgcagtgcaggccgccagtaagtatcgataactttgttttctttcacatttacaactccgacatacaaattgtaattttattactgtttggtccataaacacttgtttaccatttccttttttacaagttttaatattttctgcatatataaaacattatttattttgcagtg

SEQ ID NO: 3 - DNA, 224 bp, Artificial Sequence
  Intron1
gtaagtattcattgtaaatctgatattatttgtattattatacctacctaatttgcagtgcaggccgccagtaagtatcgataactttgttttctttcacatttacaactccgacatacaaattgtaattttattactgtttggtccataaacacttgtttaccatttccttttttacaagttttaatattttctgcatatataaaacattatttattttgcag

SEQ ID NO: 4 - DNA, 154 bp, Artificial Sequence
  Intron2
gtaagtatcgataactttgttttctttcacatttacaactccgacatacaaattgtaattttattactgtttggtccataaacacttgtttaccatttccttttttacaagttttaatattttctgcatatataaaacattatttattttgcag

SEQ ID NO: 5 - DNA, 2211 bp, Artificial Sequence
  Cap ORF
atggctgccgacggttatctacccgattggctcgaggacaaccttagtgaaggaattcgcgagtggtgggctttgaaacctggagcccctcaacccaaggcaaatcaacaacatcaagacaacgctcgaggtcttgtgcttccgggttacaaataccttggacccggcaacggactcgacaagggggagccggtcaacgcagcagacgcggcggccctcgagcacgacaaggcctacgaccagcagctcaaggccggagacaacccgtacctcaagtacaaccacgccgacgccgagttccaggagcggctcaaagaagatacgtcttttgggggcaacctcgggcgagcagtcttccaggccaaaaagaggcttcttgaacctcttggtctggttgaggaagcggctaagacggctcctggaaagaagaggcctgtagagcagtctcctcaggaaccggactcctccgcgggtattggcaaatcgggtgcacagcccgctaaaaagagactcaatttcggtcagactggcgacacagagtcagtcccagaccctcaaccaatcggagaacctcccgcagccccctcaggtgtgggatctcttacaatggcttcaggtggtggcgcaccagtggcagacaataacgaaggtgccgatggagtgggtagttcctcgggaaattggcattgcgattcccaatggctgggggacagagtcatcaccaccagcacccgaacctgggccctgcccacctacaacaatcacctctacaagcaaatctccaacagcacatctggaggatcttcaaatgacaacgcctacttcggctacagcaccccctgggggtattttgacttcaacagattccactgccacttctcaccacgtgactggcagcgactcatcaacaacaactggggattccggcctaagcgactcaacttcaagctcttcaacattcaggtcaaagaggttacggacaacaatggagtcaagaccatcgccaataaccttaccagcacggtccaggtcttcacggactcagactatcagctcccgtacgtgctcgggtcggctcacgagggctgcctcccgccgttcccagcggacgttttcatgattcctcagtacgggtatctgacgcttaatgatggaagccaggccgtgggtcgttcgtccttttactgcctggaatatttcccgtcgcaaatgctaagaacgggtaacaacttccagttcagctacgagtttgagaacgtacctttccatagcagctacgctcacagccaaagcctggaccgactaatgaatccactcatcgaccaatacttgtactatctctcaaagactattaacggttctggacagaatcaacaaacgctaaaattcagtgtggccggacccagcaacatggctgtccagggaagaaactacatacctggacccagctaccgacaacaacgtgtctcaaccactgtgactcaaaacaacaacagcgaatttgcttggcctggagcttcttcttgggctctcaatggacgtaatagcttgatgaatcctggacctgctatggccagccacaaagaaggagaggaccgtttctttcctttgtctggatctttaatttttggcaaacaaggaactggaagagacaacgtggatgcggacaaagtcatgataaccaacgaagaagaaattaaaactactaacccggtagcaacggagtcctatggacaagtggccacaaaccaccagagtgcccaagcacaggcgcagaccggctgggttcaaaaccaaggaatacttccgggtatggtttggcaggacagagatgtgtacctgcaaggacccatttgggccaaaattcctcacacggacggcaactttcacccttctccgctgatgggagggtttggaatgaagcacccgcctcctcagatcctcatcaaaaacacacctgtacctgcggatcctccaacggccttcaacaaggacaagctgaactctttcatcacccagtattctactggccaagtcagcgtggagatcgagtgggagctgcagaaggaaaacagcaagcgctggaacccggagatccagtacacttccaactattacaagtctaataatgttgaatttgctgttaatactgaaggtgtatatagtgaaccccgccccattggcaccagatacctgactcgtaatctgtaa

SEQ ID NO: 6 - DNA, 2582 bp, Artificial Sequence
  Cap gene expression cassette
atacggacctttaattcaacccaacacaatatattatagttaaataagaattattatcaaatcatttgtatattaattaaaatactatactgtaaattacattttatttacaatcactcgacgaagacttgatcacccgggggacaaggtaagtattcattgtaaatctgatattatttgtattattatacctacctaatttgcagtgcaggccgccagtaagtatcgataactttgttttctttcacatttacaactccgacatacaaattgtaattttattactgtttggtccataaacacttgtttaccatttccttttttacaagttttaatattttctgcatatataaaacattatttattttgcagtggctgccgacggttatctacccgattggctcgaggacaaccttagtgaaggaattcgcgagtggtgggctttgaaacctggagcccctcaacccaaggcaaatcaacaacatcaagacaacgctcgaggtcttgtgcttccgggttacaaataccttggacccggcaacggactcgacaagggggagccggtcaacgcagcagacgcggcggccctcgagcacgacaaggcctacgaccagcagctcaaggccggagacaacccgtacctcaagtacaaccacgccgacgccgagttccaggagcggctcaaagaagatacgtcttttgggggcaacctcgggcgagcagtcttccaggccaaaaagaggcttcttgaacctcttggtctggttgaggaagcggctaagacggctcctggaaagaagaggcctgtagagcagtctcctcaggaaccggactcctccgcgggtattggcaaatcgggtgcacagcccgctaaaaagagactcaatttcggtcagactggcgacacagagtcagtcccagaccctcaaccaatcggagaacctcccgcagccccctcaggtgtgggatctcttacaatggcttcaggtggtggcgcaccagtggcagacaataacgaaggtgccgatggagtgggtagttcctcgggaaattggcattgcgattcccaatggctgggggacagagtcatcaccaccagcacccgaacctgggccctgcccacctacaacaatcacctctacaagcaaatctccaacagcacatctggaggatcttcaaatgacaacgcctacttcggctacagcaccccctgggggtattttgacttcaacagattccactgccacttctcaccacgtgactggcagcgactcatcaacaacaactggggattccggcctaagcgactcaacttcaagctcttcaacattcaggtcaaagaggttacggacaacaatggagtcaagaccatcgccaataaccttaccagcacggtccaggtcttcacggactcagactatcagctcccgtacgtgctcgggtcggctcacgagggctgcctcccgccgttcccagcggacgttttcatgattcctcagtacgggtatctgacgcttaatgatggaagccaggccgtgggtcgttcgtccttttactgcctggaatatttcccgtcgcaaatgctaagaacgggtaacaacttccagttcagctacgagtttgagaacgtacctttccatagcagctacgctcacagccaaagcctggaccgactaatgaatccactcatcgaccaatacttgtactatctctcaaagactattaacggttctggacagaatcaacaaacgctaaaattcagtgtggccggacccagcaacatggctgtccagggaagaaactacatacctggacccagctaccgacaacaacgtgtctcaaccactgtgactcaaaacaacaacagcgaatttgcttggcctggagcttcttcttgggctctcaatggacgtaatagcttgatgaatcctggacctgctatggccagccacaaagaaggagaggaccgtttctttcctttgtctggatctttaatttttggcaaacaaggaactggaagagacaacgtggatgcggacaaagtcatgataaccaacgaagaagaaattaaaactactaacccggtagcaacggagtcctatggacaagtggccacaaaccaccagagtgcccaagcacaggcgcagaccggctgggttcaaaaccaaggaatacttccgggtatggtttggcaggacagagatgtgtacctgcaaggacccatttgggccaaaattcctcacacggacggcaactttcacccttctccgctgatgggagggtttggaatgaagcacccgcctcctcagatcctcatcaaaaacacacctgtacctgcggatcctccaacggccttcaacaaggacaagctgaactctttcatcacccagtattctactggccaagtcagcgtggagatcgagtgggagctgcagaaggaaaacagcaagcgctggaacccggagatccagtacacttccaactattacaagtctaataatgttgaatttgctgttaatactgaaggtgtatatagtgaaccccgccccattggcaccagatacctgactcgtaatctgtaa

SEQ ID NO: 7 - DNA, 92 bp, AcMNPV
  Promoter polh
atcatggagataattaaaatgataaccatctcgcaaataaataagtattttactgttttcgtaacagttttgtaataaaaaaacctataaat

SEQ ID NO: 8 - DNA, 1863 bp, Artificial Sequence
  Rep ORF
atggggttttacgagattgtgattaaggtccccagcgaccttgacgggcatctgcccggcatttctgacagctttgtgaactgggtggccgagaaggagtgggagttgccgccagattctgacttggatctgaatctgattgagcaggcacccctgaccgtggccgagaagctgcagcgcgactttctgacggagtggcgccgtgtgagtaaggccccggaggcccttttctttgtgcaatttgagaagggagagagctacttccacttacacgtgctcgtggaaaccaccggggtgaaatccttagttttgggacgtttcctgagtcagattcgcgaaaaactgattcagagaatttaccgcgggatcgagccgactttgccaaactggttcgcggtcacaaagaccagaaacggcgccggaggcgggaacaaggtggtggacgagtgctacatccccaattacttgctccccaaaacccagcctgagctccagtgggcgtggactaatttagaacagtatttaagcgcctgtttgaatctcacggagcgtaaacggttggtggcgcagcatctgacgcacgtgtcgcagacgcaggagcagaacaaagagaatcagaatcccaattctgacgcgccggtgatcagatcaaaaacttcagccaggtacatggagctggtcgggtggctcgtggacaaggggattacctcggagaagcagtggatccaggaggaccaggcctcatacatctccttcaatgcggcctccaactcgcggtcccaaatcaaggctgccttggacaatgcgggaaagattatgagcctgactaaaaccgcccccgactacctggtgggccagcagcccgtggaggacatttccagcaatcggatttataaaattttggaactaaacgggtacgatccccaatatgcggcttccgtctttctgggatgggccacgaaaaagttcggcaagaggaacaccatctggctgtttgggcctgcaactaccgggaagaccaacatcgcggaggccatagcccacactgtgcccttctacgggtgcgtaaactggaccaatgagaactttcccttcaacgactgtgtcgacaagatggtgatctggtgggaggaggggaagatgaccgccaaggtcgtggagtcggccaaagccattctcggaggaagcaaggtgcgcgtggaccagaaatgcaagtcctcggcccagatagacccgactcccgtgatcgtcacctccaacaccaacatgtgcgccgtgattgacgggaactcaacgaccttcgaacaccagcagccgttgcaagaccggatgttcaaatttgaactcacccgccgtctggatcatgactttgggaaggtcaccaagcaggaagtcaaagactttttccggtgggcaaaggatcacgtggttgaggtggagcatgaattctacgtcaaaaagggtggagccaagaaaagacccgcccccagtgacgcagatataagtgagcccaaacgggtgcgcgagtcagttgcgcagccatcgacgtcagacgcggaagcttcgatcaactacgcagacaggtaccaaaacaaatgttctcgtcacgtgggcatgaatctgatgctgtttccctgcagacaatgcgagagaatgaatcagaattcaaatatctgcttcactcacggacagaaagactgtttagagtgctttcccgtgtcagaatctcaacccgtttctgtcgtcaaaaaggcgtatcagaaactgtgctacattcatcatatcatgggaaaggtgccagacgcttgcactgcctgcgatctggtcaatgtggatttggatgactgcatctttgaacaataa

SEQ ID NO: 9 - DNA, 2220 bp, Artificial Sequence
  Rep gene expression cassette
atcatggagataattaaaatgataaccatctcgcaaataaataagtattttactgttttcgtaacagttttgtaataaaaaaacctataaatattccggattattcataccgtcccaccatcgggcgcggatccgtaagtattcattgtaaatctgatattatttgtattattatacctacctaatttgcagtgcaggccgccagtaagtatcgataactttgttttctttcacatttacaactccgacatacaaattgtaattttattactgtttggtccataaacacttgtttaccatttccttttttacaagttttaatattttctgcatatataaaacattatttattttgcagtggggttttacgagattgtgattaaggtccccagcgaccttgacgggcatctgcccggcatttctgacagctttgtgaactgggtggccgagaaggagtgggagttgccgccagattctgacttggatctgaatctgattgagcaggcacccctgaccgtggccgagaagctgcagcgcgactttctgacggagtggcgccgtgtgagtaaggccccggaggcccttttctttgtgcaatttgagaagggagagagctacttccacttacacgtgctcgtggaaaccaccggggtgaaatccttagttttgggacgtttcctgagtcagattcgcgaaaaactgattcagagaatttaccgcgggatcgagccgactttgccaaactggttcgcggtcacaaagaccagaaacggcgccggaggcgggaacaaggtggtggacgagtgctacatccccaattacttgctccccaaaacccagcctgagctccagtgggcgtggactaatttagaacagtatttaagcgcctgtttgaatctcacggagcgtaaacggttggtggcgcagcatctgacgcacgtgtcgcagacgcaggagcagaacaaagagaatcagaatcccaattctgacgcgccggtgatcagatcaaaaacttcagccaggtacatggagctggtcgggtggctcgtggacaaggggattacctcggagaagcagtggatccaggaggaccaggcctcatacatctccttcaatgcggcctccaactcgcggtcccaaatcaaggctgccttggacaatgcgggaaagattatgagcctgactaaaaccgcccccgactacctggtgggccagcagcccgtggaggacatttccagcaatcggatttataaaattttggaactaaacgggtacgatccccaatatgcggcttccgtctttctgggatgggccacgaaaaagttcggcaagaggaacaccatctggctgtttgggcctgcaactaccgggaagaccaacatcgcggaggccatagcccacactgtgcccttctacgggtgcgtaaactggaccaatgagaactttcccttcaacgactgtgtcgacaagatggtgatctggtgggaggaggggaagatgaccgccaaggtcgtggagtcggccaaagccattctcggaggaagcaaggtgcgcgtggaccagaaatgcaagtcctcggcccagatagacccgactcccgtgatcgtcacctccaacaccaacatgtgcgccgtgattgacgggaactcaacgaccttcgaacaccagcagccgttgcaagaccggatgttcaaatttgaactcacccgccgtctggatcatgactttgggaaggtcaccaagcaggaagtcaaagactttttccggtgggcaaaggatcacgtggttgaggtggagcatgaattctacgtcaaaaagggtggagccaagaaaagacccgcccccagtgacgcagatataagtgagcccaaacgggtgcgcgagtcagttgcgcagccatcgacgtcagacgcggaagcttcgatcaactacgcagacaggtaccaaaacaaatgttctcgtcacgtgggcatgaatctgatgctgtttccctgcagacaatgcgagagaatgaatcagaattcaaatatctgcttcactcacggacagaaagactgtttagagtgctttcccgtgtcagaatctcaacccgtttctgtcgtcaaaaaggcgtatcagaaactgtgctacattcatcatatcatgggaaaggtgccagacgcttgcactgcctgcgatctggtcaatgtggatttggatgactgcatctttgaacaataa

SEQ ID NO: 10 - DNA, 2358 bp, Artificial Sequence
  Cap gene expression cassette
atacggacctttaattcaacccaacacaatatattatagttaaataagaattattatcaaatcatttgtatattaattaaaatactatactgtaaattacattttatttacaatcactcgacgaagacttgatcacccggggctaagacggctgccgacggttatctacccgattggctcgaggacaaccttagtgaaggaattcgcgagtggtgggctttgaaacctggagcccctcaacccaaggcaaatcaacaacatcaagacaacgctcgaggtcttgtgcttccgggttacaaataccttggacccggcaacggactcgacaagggggagccggtcaacgcagcagacgcggcggccctcgagcacgacaaggcctacgaccagcagctcaaggccggagacaacccgtacctcaagtacaaccacgccgacgccgagttccaggagcggctcaaagaagatacgtcttttgggggcaacctcgggcgagcagtcttccaggccaaaaagaggcttcttgaacctcttggtctggttgaggaagcggctaagacggctcctggaaagaagaggcctgtagagcagtctcctcaggaaccggactcctccgcgggtattggcaaatcgggtgcacagcccgctaaaaagagactcaatttcggtcagactggcgacacagagtcagtcccagaccctcaaccaatcggagaacctcccgcagccccctcaggtgtgggatctcttacaatggcttcaggtggtggcgcaccagtggcagacaataacgaaggtgccgatggagtgggtagttcctcgggaaattggcattgcgattcccaatggctgggggacagagtcatcaccaccagcacccgaacctgggccctgcccacctacaacaatcacctctacaagcaaatctccaacagcacatctggaggatcttcaaatgacaacgcctacttcggctacagcaccccctgggggtattttgacttcaacagattccactgccacttctcaccacgtgactggcagcgactcatcaacaacaactggggattccggcctaagcgactcaacttcaagctcttcaacattcaggtcaaagaggttacggacaacaatggagtcaagaccatcgccaataaccttaccagcacggtccaggtcttcacggactcagactatcagctcccgtacgtgctcgggtcggctcacgagggctgcctcccgccgttcccagcggacgttttcatgattcctcagtacgggtatctgacgcttaatgatggaagccaggccgtgggtcgttcgtccttttactgcctggaatatttcccgtcgcaaatgctaagaacgggtaacaacttccagttcagctacgagtttgagaacgtacctttccatagcagctacgctcacagccaaagcctggaccgactaatgaatccactcatcgaccaatacttgtactatctctcaaagactattaacggttctggacagaatcaacaaacgctaaaattcagtgtggccggacccagcaacatggctgtccagggaagaaactacatacctggacccagctaccgacaacaacgtgtctcaaccactgtgactcaaaacaacaacagcgaatttgcttggcctggagcttcttcttgggctctcaatggacgtaatagcttgatgaatcctggacctgctatggccagccacaaagaaggagaggaccgtttctttcctttgtctggatctttaatttttggcaaacaaggaactggaagagacaacgtggatgcggacaaagtcatgataaccaacgaagaagaaattaaaactactaacccggtagcaacggagtcctatggacaagtggccacaaaccaccagagtgcccaagcacaggcgcagaccggctgggttcaaaaccaaggaatacttccgggtatggtttggcaggacagagatgtgtacctgcaaggacccatttgggccaaaattcctcacacggacggcaactttcacccttctccgctgatgggagggtttggaatgaagcacccgcctcctcagatcctcatcaaaaacacacctgtacctgcggatcctccaacggccttcaacaaggacaagctgaactctttcatcacccagtattctactggccaagtcagcgtggagatcgagtgggagctgcagaaggaaaacagcaagcgctggaacccggagatccagtacacttccaactattacaagtctaataatgttgaatttgctgttaatactgaaggtgtatatagtgaaccccgccccattggcaccagatacctgactcgtaatctgtaa

SEQ ID NO: 11 - DNA, 4814 bp, Artificial Sequence
  ITR -GOI
cctgcaggcagctgcgcgctcgctcgctcactgaggccgcccgggcaaagcccgggcgtcgggcgacctttggtcgcccggcctcagtgagcgagcgagcgcgcagagagggagtggccaactccatcactaggggttcctgcggccgcacgcgccgcccgtcagtgggcagagcgcacatcgcccacagtccccgagaagttggggggaggggtcggcaattgaaccggtgcctagagaaggtggcgcggggtaaactgggaaagtgatgtcgtgtactggctccgcctttttcccgagggtgggggagaaccgtatataagtgcagtagtcgccgtgaacgttctttttcgcaacgggtttgccgccagaacacgcgtaagggatccgccaccatggtgagcaagggcgaggaggataacatggccatcatcaaggagttcatgcgcttcaaggtgcacatggagggctccgtgaacggccacgagttcgagatcgagggcgagggcgagggccgcccctacgagggcacccagaccgccaagctgaaggtgaccaagggtggccccctgcccttcgcctgggacatcctgtcccctcagttcatgtacggctccaaggcctacgtgaagcaccccgccgacatccccgactacttgaagctgtccttccccgagggcttcaagtgggagcgcgtgatgaacttcgaggacggcggcgtggtgaccgtgacccaggactcctccctgcaggacggcgagttcatctacaaggtgaagctgcgcggcaccaacttcccctccgacggccccgtaatgcagaagaagaccatgggctgggaggcctcctccgagcggatgtaccccgaggacggcgccctgaagggcgagatcaagcagaggctgaagctgaaggacggcggccactacgacgctgaggtcaagaccacctacaaggccaagaagcccgtgcagctgcccggcgcctacaacgtcaacatcaagttggacatcacctcccacaacgaggactacaccatcgtggaacagtacgaacgcgccgagggccgccactccaccggcggcatggacgagctgtacaagtaagaattcgatatcaagcttatcgataatcaacctctggattacaaaatttgtgaaagattgactggtattcttaactatgttgctccttttacgctatgtggatacgctgctttaatgcctttgtatcatgctattgcttcccgtatggctttcattttctcctccttgtataaatcctggttgctgtctctttatgaggagttgtggcccgttgtcaggcaacgtggcgtggtgtgcactgtgtttgctgacgcaacccccactggttggggcattgccaccacctgtcagctcctttccgggactttcgctttccccctccctattgccacggcggaactcatcgccgcctgccttgcccgctgctggacaggggctcggctgttgggcactgacaattccgtggtgttgtcggggaaatcatcgtcctttccttggctgctcgcctgtgttgccacctggattctgcgcgggacgtccttctgctacgtcccttcggccctcaatccagcggaccttccttcccgcggcctgctgccggctctgcggcctcttccgcgtcttcgccttcgccctcagacgagtcggatctccctttgggccgcctccccgcatcgataccgagcgctgctcgagagatctacgggtggcatccctgtgacccctccccagtgcctctcctggccctggaagttgccactccagtgcccaccagccttgtcctaataaaattaagttgcatcattttgtctgactaggtgtccttctataatattatggggtggaggggggtggtatggagcaaggggcaagttgggaagacaacctgtagggcctgcggggtctattgggaaccaagctggagtgcagtggcacaatcttggctcactgcaatctccgcctcctgggttcaagcgattctcctgcctcagcctcccgagttgttgggattccaggcatgcatgaccaggctcagctaatttttgtttttttggtagagacggggtttcaccatattggccaggctggtctccaactcctaatctcaggtgatctacccaccttggcctcccaaattgctgggattacaggcgtgaaccactgctcccttccctgtccttctgattttgtaggtaaccacgtgcggaccgagcggccgcaggaacccctagtgatggagttggccactccctctctgcgcgctcgctcgctcactgaggccgggcgaccaaaggtcgcccgacgcccgggctttgcccgggcggcctcagtgagcgagcgagcgcgcagctgcctgcaggcctgcaggcagctgcgcgctcgctcgctcactgaggccgcccgggcaaagcccgggcgtcgggcgacctttggtcgcccggcctcagtgagcgagcgagcgcgcagagagggagtggccaactccatcactaggggttcctgcggccgcacgcgccgcccgtcagtgggcagagcgcacatcgcccacagtccccgagaagttggggggaggggtcggcaattgaaccggtgcctagagaaggtggcgcggggtaaactgggaaagtgatgtcgtgtactggctccgcctttttcccgagggtgggggagaaccgtatataagtgcagtagtcgccgtgaacgttctttttcgcaacgggtttgccgccagaacacgcgtaagggatccgccaccatggtgagcaagggcgaggaggataacatggccatcatcaaggagttcatgcgcttcaaggtgcacatggagggctccgtgaacggccacgagttcgagatcgagggcgagggcgagggccgcccctacgagggcacccagaccgccaagctgaaggtgaccaagggtggccccctgcccttcgcctgggacatcctgtcccctcagttcatgtacggctccaaggcctacgtgaagcaccccgccgacatccccgactacttgaagctgtccttccccgagggcttcaagtgggagcgcgtgatgaacttcgaggacggcggcgtggtgaccgtgacccaggactcctccctgcaggacggcgagttcatctacaaggtgaagctgcgcggcaccaacttcccctccgacggccccgtaatgcagaagaagaccatgggctgggaggcctcctccgagcggatgtaccccgaggacggcgccctgaagggcgagatcaagcagaggctgaagctgaaggacggcggccactacgacgctgaggtcaagaccacctacaaggccaagaagcccgtgcagctgcccggcgcctacaacgtcaacatcaagttggacatcacctcccacaacgaggactacaccatcgtggaacagtacgaacgcgccgagggccgccactccaccggcggcatggacgagctgtacaagtaagaattcgatatcaagcttatcgataatcaacctctggattacaaaatttgtgaaagattgactggtattcttaactatgttgctccttttacgctatgtggatacgctgctttaatgcctttgtatcatgctattgcttcccgtatggctttcattttctcctccttgtataaatcctggttgctgtctctttatgaggagttgtggcccgttgtcaggcaacgtggcgtggtgtgcactgtgtttgctgacgcaacccccactggttggggcattgccaccacctgtcagctcctttccgggactttcgctttccccctccctattgccacggcggaactcatcgccgcctgccttgcccgctgctggacaggggctcggctgttgggcactgacaattccgtggtgttgtcggggaaatcatcgtcctttccttggctgctcgcctgtgttgccacctggattctgcgcgggacgtccttctgctacgtcccttcggccctcaatccagcggaccttccttcccgcggcctgctgccggctctgcggcctcttccgcgtcttcgccttcgccctcagacgagtcggatctccctttgggccgcctccccgcatcgataccgagcgctgctcgagagatctacgggtggcatccctgtgacccctccccagtgcctctcctggccctggaagttgccactccagtgcccaccagccttgtcctaataaaattaagttgcatcattttgtctgactaggtgtccttctataatattatggggtggaggggggtggtatggagcaaggggcaagttgggaagacaacctgtagggcctgcggggtctattgggaaccaagctggagtgcagtggcacaatcttggctcactgcaatctccgcctcctgggttcaagcgattctcctgcctcagcctcccgagttgttgggattccaggcatgcatgaccaggctcagctaatttttgtttttttggtagagacggggtttcaccatattggccaggctggtctccaactcctaatctcaggtgatctacccaccttggcctcccaaattgctgggattacaggcgtgaaccactgctcccttccctgtccttctgattttgtaggtaaccacgtgcggaccgagcggccgcaggaacccctagtgatggagttggccactccctctctgcgcgctcgctcgctcactgaggccgggcgaccaaaggtcgcccgacgcccgggctttgcccgggcggcctcagtgagcgagcgagcgcgcagctgcctgcagg

SEQ ID NO: 12 - DNA, 2579 bp, Artificial Sequence
  Cap gene expression cassette
atacggacctttaattcaacccaacacaatatattatagttaaataagaattattatcaaatcatttgtatattaattaaaatactatactgtaaattacattttatttacaatcactcgacgaagacttgatcacccgggggacaaggtaagtattcattgtaaatctgatattatttgtattattatacctacctaatttgcagtgcaggccgccagtaagtatcgataactttgttttctttcacatttacaactccgacatacaaattgtaattttattactgtttggtccataaacacttgtttaccatttccttttttacaagttttaatattttctgcatatataaaacattatttattttgcagtggctgccgacggttatctacccgattggctcgaggacactctctctgaaggaataagacagtggtggaagctcaaacctggcccaccaccaccaaagcccgcagagcggcataaggacgacagcaggggtcttgtgcttcctgggtacaagtacctcggacccttcaacggactcgacaagggagagccggtcaacgaggcagacgccgcggccctcgagcacgacaaagcctacgaccggcagctcgacagcggagacaacccgtacctcaagtacaaccacgccgacgcggagtttcaggagcgccttaaagaagatacgtcttttgggggcaacctcggacgagcagtcttccaggcgaaaaagagggttcttgaacctctgggcctggttgaggaacctgttaagacggctccgggaaaaaagaggccggtagagcactctcctgtggagccagactcctcctcgggaaccggaaaggcgggccagcagcctgcaagaaaaagattgaattttggtcagactggagacgcagactcagtacctgacccccagcctctcggacagccaccagcagccccctctggtctgggaactaatacgatggctacaggcagtggcgcaccaatggcagacaataacgagggcgccgacggagtgggtaattcctcgggaaattggcattgcgattccacatggatgggcgacagagtcatcaccaccagcacccgaacctgggccctgcccacctacaacaaccacctctacaaacaaatttccagccaatcaggagcctcgaacgacaatcactactttggctacagcaccccttgggggtattttgacttcaacagattccactgccacttttcaccacgtgactggcaaagactcatcaacaacaactggggattccgacccaagagactcaacttcaagctctttaacattcaagtcaaagaggtcacgcagaatgacggtacgacgacgattgccaataaccttaccagcacggttcaggtgtttactgactcggagtaccagctcccgtacgtcctcggctcggcgcatcaaggatgcctcccgccgttcccagcagacgtcttcatggtgccacagtatggatacctcaccctgaacaacgggagtcaggcagtaggacgctcttcattttactgcctggagtactttccttctcagatgctgcgtaccggaaacaactttaccttcagctacacttttgaggacgttcctttccacagcagctacgctcacagccagagtctggaccgtctcatgaatcctctcatcgaccagtacctgtattacttgagcagaacaaacactccaagtggaaccaccacgcagtcaaggcttcagttttctcaggccggagcgagtgacattcgggaccagtctaggaactggcttcctggaccctgttaccgccagcagcgagtatcaaagacatctgcggataacaacaacagtgaatactcgtggactggagctaccaagtaccacctcaatggcagagactctctggtgaatccgggcccggccatggcaagccacaaggacgatgaagaaaagttttttcctcagagcggggttctcatctttgggaagcaaggctcagagaaaacaaatgtggacattgaaaaggtcatgattacagacgaagaggaaatcaggacaaccaatcccgtggctacggagcagtatggttctgtatctaccaacctccagagaggcaacagacaagcagctaccgcagatgtcaacacacaaggcgttcttccaggcatggtctggcaggacagagatgtgtaccttcaggggcccatctgggcaaagattccacacacggacggacattttcacccctctcccctcatgggtggattcggacttaaacaccctcctccacagattctcatcaagaacaccccggtacctgcgaatccttcgaccaccttcagtgcggcaaagtttgcttccttcatcacacagtactccacgggacaggtcagcgtggagatcgagtgggagctgcagaaggaaaacagcaaacgctggaatcccgaaattcagtacacttccaactacaacaagtctgttaatgtggactttactgtggacactaatggcgtgtattcagagcctcgccccattggcaccagatacctgactcgtaatctgtaa

SEQ ID NO: 13 - DNA, 2546 bp, Artificial Sequence
  Cap gene expression cassette
atacggacctttaattcaacccaacacaatatattatagttaaataagaattattatcaaatcatttgtatattaattaaaatactatactgtaaattacattttatttacaatcactcgacgaagacttgatcacccgggggacaaggtaagtattcattgtaaatctgatattatttgtattattatacctacctaatttgcagtgcaggccgccagtaagtatcgataactttgttttctttcacatttacaactccgacatacaaattgtaattttattactgtttggtccataaacacttgtttaccatttccttttttacaagttttaatattttctgcatatataaaacattatttattttgcagtgtcttttgttgatcacccacccgattggttggaagaagttggtgaaggtcttcgcgagtttttgggccttgaagcgggcccaccgaaaccaaaacccaatcagcagcatcaagatcaagcccgtggtcttgtgctgcctggttataactatctcggacccggaaacggtctcgatcgaggagagcctgtcaacagggcagacgaggtcgcgcgagagcacgacatctcgtacaacgagcagcttgaggcgggagacaacccctacctcaagtacaaccacgcggacgccgagtttcaggagaagctcgccgacgacacatccttcgggggaaacctcggaaaggcagtctttcaggccaagaaaagggttctcgaaccttttggcctggttgaagagggtgctaagacggcccctaccggaaagcggatagacgaccactttccaaaaagaaagaaggctcggaccgaagaggactccaagccttccacctcgtcagacgccgaagctggacccagcggatcccagcagctgcaaatcccagcccaaccagcctcaagtttgggagctgatacaatgtctgcgggaggtggcggcccattgggcgacaataaccaaggtgccgatggagtgggcaatgcctcgggagattggcattgcgattccacgtggatgggggacagagtcgtcaccaagtccacccgaacctgggtgctgcccagctacaacaaccaccagtaccgagagatcaaaagcggctccgtcgacggaagcaacgccaacgcctactttggatacagcaccccctgggggtactttgactttaaccgcttccacagccactggagcccccgagactggcaaagactcatcaacaactactggggcttcagaccccggtccctcagagtcaaaatcttcaacattcaagtcaaagaggtcacggtgcaggactccaccaccaccatcgccaacaacctcacctccaccgtccaagtgtttacggacgacgactaccagctgccctacgtcgtcggcaacgggaccgagggatgcctgccggccttccctccgcaggtctttacgctgccgcagtacggttacgcgacgctgaaccgcgacaacacagaaaatcccaccgagaggagcagcttcttctgcctagagtactttcccagcaagatgctgagaacgggcaacaactttgagtttacctacaactttgaggaggtgcccttccactccagcttcgctcccagtcagaacctcttcaagctggccaacccgctggtggaccagtacttgtaccgcttcgtgagcacaaataacactggcggagtccagttcaacaagaacctggccgggagatacgccaacacctacaaaaactggttcccggggcccatgggccgaacccagggctggaacctgggctccggggtcaaccgcgccagtgtcagcgccttcgccacgaccaataggatggagctcgagggcgcgagttaccaggtgcccccgcagccgaacggcatgaccaacaacctccagggcagcaacacctatgccctggagaacactatgatcttcaacagccagccggcgaacccgggcaccaccgccacgtacctcgagggcaacatgctcatcaccagcgagagcgagacgcagccggtgaaccgcgtggcgtacaacgtcggcgggcagatggccaccaacaaccagagctccaccactgcccccgcgaccggcacgtacaacctccaggaaatcgtgcccggcagcgtgtggatggagagggacgtgtacctccaaggacccatctgggccaagatcccagagacgggggcgcactttcacccctctccggccatgggcggattcggactcaaacacccaccgcccatgatgctcatcaagaacacgcctgtgcccggaaatatcaccagcttctcggacgtgcccgtcagcagcttcatcacccagtacagcaccgggcaggtcaccgtggagatggagtgggagctcaagaaggaaaactccaagaggtggaacccagagatccagtacacaaacaactacaacgacccccagtttgtggactttgccccggacagcaccggggaatacagaagcaccagacctatcggaacccgataccttacccgacccctttaa

SEQ ID NO: 14 - DNA, 2588 bp, Artificial Sequence
  Cap gene expression cassette
atacggacctttaattcaacccaacacaatatattatagttaaataagaattattatcaaatcatttgtatattaattaaaatactatactgtaaattacattttatttacaatcactcgacgaagacttgatcacccgggggacaaggtaagtattcattgtaaatctgatattatttgtattattatacctacctaatttgcagtgcaggccgccagtaagtatcgataactttgttttctttcacatttacaactccgacatacaaattgtaattttattactgtttggtccataaacacttgtttaccatttccttttttacaagttttaatattttctgcatatataaaacattatttattttgcagtggctgccgacggttatctacccgattggctcgaggacaacctctctgagggcattcgcgagtggtgggcgctgaaacctggagccccgaagcccaaagccaaccagcaaaagcaggacgacggccggggtctggtgcttcctggctacaagtacctcggacccttcaacggactcgacaagggggagcccgtcaacgcggcggacgcagcggccctcgagcacgacaaggcctacgaccagcagctgcaggcgggtgacaatccgtacctgcggtataaccacgccgacgccgagtttcaggagcgtctgcaagaagatacgtcttttgggggcaacctcgggcgagcagtcttccaggccaagaagcgggttctcgaacctctcggtctggttgaggaaggcgctaagacggctcctggaaagaagagaccggtagagccatcaccccagcgttctccagactcctctacgggcatcggcaagaaaggccaacagcccgccagaaaaagactcaattttggtcagactggcgactcagagtcagttccagaccctcaacctctcggagaacctccagcagcgccctctggtgtgggacctaatacaatggctgcaggcggtggcgcaccaatggcagacaataacgaaggcgccgacggagtgggtagttcctcgggaaattggcattgcgattccacatggctgggcgacagagtcatcaccaccagcacccgaacctgggccctgcccacctacaacaaccacctctacaagcaaatctccaacgggacatcgggaggagccaccaacgacaacacctacttcggctacagcaccccctgggggtattttgactttaacagattccactgccacttttcaccacgtgactggcagcgactcatcaacaacaactggggattccggcccaagagactcagcttcaagctcttcaacatccaggtcaaggaggtcacgcagaatgaaggcaccaagaccatcgccaataacctcaccagcaccatccaggtgtttacggactcggagtaccagctgccgtacgttctcggctctgcccaccagggctgcctgcctccgttcccggcggacgtgttcatgattccccagtacggctacctaacactcaacaacggtagtcaggccgtgggacgctcctccttctactgcctggaatactttccttcgcagatgctgagaaccggcaacaacttccagtttacttacaccttcgaggacgtgcctttccacagcagctacgcccacagccagagcttggaccggctgatgaatcctctgattgaccagtacctgtactacttgtctcggactcaaacaacaggaggcacggcaaatacgcagactctgggcttcagccaaggtgggcctaatacaatggccaatcaggcaaagaactggctgccaggaccctgttaccgccaacaacgcgtctcaacgacaaccgggcaaaacaacaatagcaactttgcctggactgctgggaccaaataccatctgaatggaagaaattcattggctaatcctggcatcgctatggcaacacacaaagacgacgaggagcgtttttttcccagtaacgggatcctgatttttggcaaacaaaatgctgccagagacaatgcggattacagcgatgtcatgctcaccagcgaggaagaaatcaaaaccactaaccctgtggctacagaggaatacggtatcgtggcagataacttgcagcagcaaaacacggctcctcaaattggaactgtcaacagccagggggccttacccggtatggtctggcagaaccgggacgtgtacctgcagggtcccatctgggccaagattcctcacacggacggcaacttccacccgtctccgctgatgggcggctttggcctgaaacatcctccgcctcagatcctgatcaagaacacgcctgtacctgcggatcctccgaccaccttcaaccagtcaaagctgaactctttcatcacgcaatacagcaccggacaggtcagcgtggaaattgaatgggagctgcagaaggaaaacagcaagcgctggaaccccgagatccagtacacctccaactactacaaatctacaagtgtggactttgctgttaatacagaaggcgtgtactctgaaccccgccccattggcacccgttacctcacccgtaatctgtaa